European Patent Application EP 4 751 775 A1, published June 3, 2026. Title: N-CARBAMOYL SYDNONE IMINES FOR USE IN THE TREATMENT OF FLAVIVIRUS INFECTIONS. Applicant: IRBM S.p.A. Application EP. The sequence listing filed with the application follows.

SEQUENCE LISTING (3 sequences)

SEQ ID NO: 1 - protein, 247 aa, Zika virus
MGSSHHHHHHSSGLVPRGSHMVDMYIERAGDITWEKDAEVTGNSPRLDVALDESGDFSLVEDDGPPMAGGGGSGGGGSGALWDVPAPKEVKKGETTDGVYRVMTRGLLGSTQVGVGVMQEGVFHTMWHVTKGSALRSGEGRLDPYWGDVKQDLVSYCGPWKLDAAWDGHSEVQLLAVPPGERARNIQTLPGIFKTKDGDIGAVALDYPAGTSGSPILDKCGRVIGLYGNGVVIKNGSYVSAITQGRR

SEQ ID NO: 2 - protein, 7 aa, West Nile virus
MHHHHHH

SEQ ID NO: 3 - protein, 9 aa, West Nile virus
GGGGSGGGG